European Patent Application EP 4 667 560 A1, published December 24, 2025. Title: GABA-producing Levilactobacillus brevis strain and its use. Applicant: Evonik Operations GmbH. The sequence listing filed with the application follows.

SEQUENCE LISTING (6 sequences)

SEQ ID NO: 1 - DNA, 1566 bp, Levilactobacillus brevis
  source 1..1566: mol_type = genomic DNA
taagatgagagtttgatcctggctcaggacgaacgctggcggcatgcctaatacatgcaagtcgaacgagcttccgttgaatgacgtgcttgcactgatttcaacaatggagcgagtggcgaactggtgagtaacacgtggggaatctgcccagaagcaggggataacacttggaaacaggtgctaataccgtataacaacaaaatccgcatggattttgtttgaaaggtggcttcggctatcacttctggatgatcccgcggcgtattagttagttggtgaggtaaaggcccaccaagacgatgatacgtagccgacctgagagggtaatcggccacattgggactgagacacggcccaaactcctacgggaggcagcagtagggaatcttccacaatggacgaaagtctgatggagcaatgccgcgtgagtgaagaagggtttcggctcgtaaaactctgttgttaaagaagaacacctttgagagtaactgttcaagggttgacggtatttaaccagaaagccacggctaactacgtgccagcagccgcggtaatacgtaggtggcaagcgttgtccggatttattgggcgtaaagcgagcgcaggcggttttttaagtctgatgtgaaagccttcggcttaaccggagaagtgcatcggaaactgggagacttgagtgcagaagaggacagtggaactccatgtgtagcggtggaatgcgtagatatatggaagaacaccagtggcgaaggcggctgtctagtctgtaactgacgctgaggctcgaaagcatgggtagcgaacaggattagataccctggtagtccatgccgtaaacgatgagtgctaagtgttggagggtttccgcccttcagtgctgcagctaacgcattaagcactccgcctggggagtacgaccgcaaggttgaaactcaaaggaattgacgggggcccgcacaagcggtggagcatgtggtttaattcgaagctacgcgaagaaccttaccaggtcttgacatcttctgccaatcttagagataagacgttcccttcggggacagaatgacaggtggtgcatggttgtcgtcagctcgtgtcgtgagatgttgggttaagtcccgcaacgagcgcaacccttattatcagttgccagcattcagttgggcactctggtgagactgccggtgacaaaccggaggaaggtggggatgacgtcaaatcatcatgccccttatgacctgggctacacacgtgctacaatggacggtacaacgagttgcgaagtcgtgaggctaagctaatctcttaaagccgttctcagttcggattgtaggctgcaactcgcctacatgaagttggaatcgctagtaatcgcggatcagcatgccgcggtgaatacgttcccgggccttgtacacaccgcccgtcacaccatgagagtttgtaacacccaaagccggtgagataaccttcgggagtcagccgtctaaggtgggacagatgattagggtgaagtcgtaacaaggtagccgtaggagaacctgcggctggatcacctccttt

SEQ ID NO: 2 - DNA, 3612 bp, Levilactobacillus brevis
  source 1..3612: mol_type = genomic DNA
ttggcaggacacttagtgaaatacgggaaacaccgtacgcgccggagctattcgcgaatcaaggaagttcttgatttacctaacttgattgagattcaaaccaattcctataattggttccttgacgaaggtttacgcgatatgttcgacgacatcatgccaatcgaagattttcaaggaaacctttcgttagagtttgttgattatcagttactagaacccaaatacagcgtggatgaagcacgggaacatgatgccaactactcggcaccgctacacgtcaccctgcggttaaccaaccacgaaacgggtgaaatcaaatcacaagacgtcttctttggtgactttccattaatgacggcccaagggaccttcattattaacggggcggaacgggttattgtttctcaattagtccgttcaccaggggtttacttcaatgaagatacggataagaacggtcggacagtttacggtgccactgtgatccctaaccggggtgcatggctagaatttgaaactgatgcgaagaacgtttcttacgttcggattgaccggacgcggaagatcccaatgaccgaattagttcgggccttagggtttggttctgacgatgaaatcttagatatcttaggtgacaacgaaagcttgatgcagacgttggaaaaggatatccataagaacaccgatgactcacgtgtcgaagagtccttgaaggatatctacgaacgcttgcgtccaggtgaacctaagacggcggactcttcacggagtttgctgactgctcggttcttcgatcctaaacgctatgacatggcaccagttggtcgttacaagactaacaagaagctgagtttaaagacccgtttgctgggcttgaccttagctgaaacgttggctgatcctgataccggtgaaattattgccgctaaaggaacggtcgttgacaaggacgtgatgaagagcttagcaccattcttggatcaagatgatttcaagatggtgactttccaaccttctgacgaagccgttgtcacggaaccactaaaattacaaattatcaaagtacaatcaccagatgatccagaacaagaagttcctgtgattgggaatgggaacatcgatatcaagctgaagcacattcgtccagccgatattattgcatccatgaactacttctttgacttacaactggggattggtaacactgatgatattgaccacttggggaaccgacggattcgttccgttggtgaattactccaaaaccaattccggatcgggttatcccggatggaacgggttgttcgtgaacggatgtccattcaagatgctgcgacggtaacgccacaacaattgattaacattcgtcctgtcgtggcctcaattaaagaattctttgggtcttcacagttgtctcaattcatggatcagactaacccgttaggtgaattaacgcataaacggcgtctgtctgctttgggacctggtgggttaacgcgtgaccgggccggttatgaagtccgggacgtgcactatacccattatggtcggatgtgcccaattgaaacgcctgaagggcctaacattgggttgatcaacagtttgtccagctatgcccgggttaacaagtatgggttcatcgagacgccataccgtcgtgtttcttgggatacgcataaggttaccgataagatcgattacctgacagctgatgaagaagataactatgttgttgctcaggccaacacgccattaaatgatgatggttccttcaatacggatacgatcatggcccgtgcccaatctgaaaacattgaaaccagtgctgaccggattgactacatggatgtttcgcctaagcaagttgttgcggttgccacggcatgtattcctttcttggaaaacgatgactccaaccgggccctgatgggtgccaacatgcaacggcaagctgtgccattgttgaacccacatgcgccattaattggtactgggattgaatacaaagcggcccatgactcaggggttgctttgatcagtcaacatgatgggactgttgaatacgttgatgcacgtgaaattcgtgttcggcgtgaagatggtgccttagacacttacaagctcatgaagttccgccggtcaaacggtgggaagaactacaaccaacgcccaatcgttaaggtcggcgaccatgtcgataacgatgaagtcttggctgatggtccttccatggaaaatggggaattggctttgggtcaaaacccattagttgccttcatgacttggcaagggtacaacttcgaagatgccattgggatcaacgagcggttggttcgcgatgacgtttacacgtcgattcatattgaagaatacgaatcagaagcgcgtgatacgaagcttggacctgaagaaatgacgcgtgaaattcctaacgttggggaagatgccttgaagaacttggacgaagacgggattatccgtgttggtgccgaagttcaagatggggatatcttagttggtaaggtaacgcctaagggtgttactgaattatccgctgaggaacgactccttcatgccatctttggtgaaaaggcccgtgaagttcgggatacttctctgaaggtaccgcatggtggtggcgggatcatccaagatgtgaagatctttacccgtgaaaatggggacgaattgtcaccaggtgtcaacatgatggttcgggtctacatcgcgcaaaagcggaagatccaagttggggacaagatgtctggacgtcacggtaacaaggggacggtttcagtggttatccctgaagaagatatgccgtacatgccagatggtaccccaatcgacattatgttgagtcccatgggtgtgccttcccggatgaacatcgggcaagtgctcgaattgcatttggggatggctgctcgcaagctcggtgtgcacatggcaaccccagtctttgatggtgcccaagatacagatattgcggacgctgttaaggaagccgggatggctgctgacgccaagactgtcttatatgatggtcgaactggtgaaccgtttgataagcgggttgccgttggggtcatgcactacctgaagttggcccacatggttgatgacaagatgcacgcccgttctatcggaccttactcactggttacgcaacaaccccttggtgggaaagcgcaatttggtggtcagcgtttcggtgaaatggaagtttgggctttggaagcttatggtgccgcttatacgttgcaagaaatcttgacgtacaagtctgatgacgtggttggtcgggttaagacctacgaagccattgttaagggcgatccaattccaaagccaggtgttcctgaatccttccgcgtgttagtgaaggaactccaatccttagggctggacatgaaggtcttaaatggcgacaaagaagaaatcgaactccgtgatatggacgacgaagacgacgatgttgttaatgtggatgcgttgagcaagtacgcgcaacaacaggaagaacaacggaaagccgctgctcagactgatgaatccaagaccgcgccagcaacaaaaaatgaaagtcaaccgaatacacaagactaa

SEQ ID NO: 3 - DNA, 1944 bp, Levilactobacillus brevis
  source 1..1944: mol_type = genomic DNA
gtggcagacgaaaaagaaaccaaagcgcaacaagctcgtgagtatgacgccagtcaaattcaagtcttggaaggtttggaagcggtccggaaacggcccgggatgtacattggctcgacgagttcccaagggttacaccatttagtttgggaaattgtcgataacgggattgatgaggccttagcaggctttgctgatgaaatccacgtgacagtcaaccaagacaacagcattaccgttaccgataacggtcggggaattccgattggtatccaaaagaagacgggaaaaccagcgttagaaactgttttcacgattctgcatgccggtggtaaattcggcggtggcggatataaggtttctggtggtcttcatggggtgggtgcttccgtagttaacgccttgtctactgatcttgaggcgcaagtgacacgtgatggcaagacctatgcgattgcctttgaccacggccacgttaagacgccaatgcacgtgattaaagagggcctgccacaagaccaacacgggacggcagttcactttttaccggacccagatattttccgagaaacgaccgtctttgatattaagacattgacgacgcggattcgggaactggccttcttaaacaaaggcttgcggattactattcgtgatgaacgtccggaaaagccaacggaagaagatttcctttacgaaggcggtatccggcattacgtagactatttgaacgaaaacaaagaaacgttatttgaaccgccaatttacgtggaagggcaagaaaacggtattacggtggaagtcgcgttgcaatacacggacgactaccacaataacctcttaactttcaccaacaacatccacacctatgaaggtgggacccatgaagaagggttcaaacgggcgttgacgcgggttgtgaatgattatgcccggcaaaacaagttgatgaaagataatgaagccaacttgaccggggatgatgtccgtgaagggttgacagctgtggtttccgtgaagcatccggatccgcaatttgaaggtcaaacgaagaccaaattagggaactctgatgcccgcacggctgtcgatcacacctttgctgaccactttatgcggttcatgatggaacatccagatgtcgcccggaagattgtggacaaagggacgctggcgtctaaagcacgtgttgctgctaaacgggcccgtgaagtgacgcggaagaagagcggcctggaaatcagcaatttacctggtaagttagctgataacacgtctaaagatcccgaaatctctgaactctttatcgtcgaaggggattctgctggtgggtctgccaagcaaggtcgttcgcggctgacgcaggccattctgccaattcgggggaagattttaaacgtggaaaaggcgtcgatggaccggatcttagcaaacgaagaaattcggtcactctttacggctatgggaacgggttttggtaatgactttgatgtgtctaaggtaaattaccacaagcttattttgatgaccgatgccgatgtcgatggtgcgcacattcggacgctgttgttgacgctggtttaccgctacatgcggccattattggatgctggctttgtctatattgcctgcccaccgctttatcgagttcgccagggtaagatgcaacggtacttggattctgatgaagaattaaaggatctgttggggcaattgccaccatcaccaaaaccacaaatccaacggtataaagggttaggggaaatggacgcggaacaattgtgggaaacgaccatgaacccagaaaaccggcggctcttgcgggttgatgcgcaagatgccatcaatgccgatcaagtctttacgatgttgatgggcgataaggtggccccacggcgtgagtttatcgaaaataacgccacgtttgccgaactggatgtttag

SEQ ID NO: 4 - DNA, 1455 bp, Levilactobacillus brevis
  source 1..1455: mol_type = genomic DNA
atgggattatttgatattttccggcggcgagcgaaagaaacaccagctagccaagcggaagaaacaccagttgagtcgaccgcaacaacgtctactgccgccagtgaagcgagcgaatcggcagctgataacgctacgtcagttgctagtgaagcatctgccgcagcagaaaccagcgaggttgctgaatcaacagtagctggttcagtaccggttgctaacagcgattcagcagatactaatgcatcactggcagcgaccgctactagcgatgcagcggttgaaactgaaacgagcgaaacgtctcgtgcagattcggcatcagtaacagctgatgtcttagatagtgtggcatcggcaactagcgcagcagcgacagttgatacgccaaccgaagtgctacagtcaacaccgccagcctcatcagcatctgctgaggtagagacgcctgcaacaaccgtcgaagagtcttcgacaactgacgcctcggcaccagaagcaagtgatgagcaactttatgacaaagggttggaaaaaacccggacgacttttggccaacgactgaatgccttattggctaatttccggcacgttgacgagagtttctttgatgacttggaagagacgttaatcggagccgatgtcgggtttgatatggcggttaaactcagtgatgagttgcgtgacgaggttaagttacaaaacgcgaaaaagtcacaggatgttcaaaacgtagtggttgaaaagctggtggagatttatgaggcagccggtaatcatgaaactacggctatcaatatggcagaaaccgggccaacggtgatcctattcgttggggtcaatggcgtggggaagacgaccaccatcggcaaaatggctaatcgttatcatcaggcgggcaagaaagtcttactggcggcggcggatacgtttagagctggtgcaactgaacaacttgatgtgtgggctaaacgcgcggatgttgatattgtgacgggaaagccacagtcagatcccgcagcggttgtttttgatgctgttcaaaaggctaagcaagatgattatgacattttgtttgttgatacggctggtcggctacaaaacaaggtcaacttgatgaatgaattggaaaagatgaagcggatcattacgcgagaaattccaagtgccccacatgaggtcttgttggtgttagatgccacaacgggtcaaaacgcgttaacacaagctaagctgtttaaggagtccacggcagtaacggggattgtcttgaccaagcttgatggaacggctcgggggggaattgttctggccattcgtaacgagttacacgtgccagtcaagttcattggtttaggtgagcagatttctgacttgcggccatttgacccgaacgagtttgtttatgggttatttaaagggttgattgatgtgaaggctttagataataaataa

SEQ ID NO: 5 - DNA, 1101 bp, Levilactobacillus brevis
  source 1..1101: mol_type = genomic DNA
atgtcattaactgcaggaatcgttgggctgcctaacgtcggtaagtccacgttatttaacgccatcacgaaggccggcgccgaaatggccaactacccattcgccacgatcgatccaaatgtgggcatggtcgaagtgcctgataaccggttggatcggattcaagaactgatcccagcgaaaaaagttgtgccaaccacctttgaatttacggatattgccgggatcgtcaagggggccagcaagggtgaaggactgggtaaccagttcttggaaaacattcgccaagtggacgccatcgttcacgttgtccgggcctttgatgacgacaacattacccacgtctccggtaaaattgatcccatcgatgatattgaaaccattaatttggaacttggtttgtctgacttagaagccgttaacaaacggttggctaaggttgaacgggctgctaaggggagcgacaaggaagctaaggctgaattggccgttttgcaaaagattaagccggttctcgaagccggcggtgccgtgcggacaattgactttgacgaagaagaaatgaagatcgtcaagggcttgttcttactgacatccaagccagtcttgtacgtggctaacattgccgaagacgacatggctgatcccgaagactctaagtactttgggttaatcaaggactatgcggctaaggaaggcgccgaggccattgctgtggccgctgaagctgaagaagaaattgcacagttagatgatgacgagaagcaagacttcttggaagctgaaggcgtcgaagaacccggcttgaaccggctaattcgggcgtcatatcatctcttaggcttacaaacgttcttcacggctggtggtaaggaaacacgggcgtggacgtttaaaacggggactaaggcccctcaagcggctggtattattcactccgacttcgaacgaggcttcattcgtgccgaagtcatggcctttgcggatttggatcaatttgaatccgaagcagcggtgaaggaagccggtaaactccgagttgaagggaaagactacgtgatggaagacggcgatatcgtcgaattccgattcaacgtttag

SEQ ID NO: 6 - DNA, 693 bp, Levilactobacillus brevis
  source 1..693: mol_type = genomic DNA
ttgcgtacgaccgccaaggtattagtcgtggaggatgagaaggcattatccgcagacattgttgagttaatcgaaccgatttgtgaaacaacaacagctttcgatggtgagcaaggagaatttttggcaagtcagggcgtctttgacgctattattttggacctgatgttaccaggtgaaagtgggttggatctcttgctccacatccgcaaccagggggtcaagacaccggtgttgattctaaccgctaaagataccattgctgataagttacgcggctttaatgacggtgcggatgactatgtgactaagccctttcaccgagaagaattattagcgcgaatgaaggctctgttaaaacggactggtcatctgaatagtagtgatacgattgcgctgggacaactggaaattaacaccagtaaacatctggccacctttaatggcgcaccactgacgttaaaggggcgggaatttgatttgctagcttacttagtagggaatccagggaccattattaccaaggaacaaatcttcaatcggctctggggatttgattccgagaccagcctttccgtggttgaagtgtatatgagtaacctgagaaaggagctcaaacacgctggcagtgatctgtcattacgaacgattcgtaatgcgggttacattgtggaggccccagatgagcaataa